European Patent Application EP 4 755 904 A2, published June 10, 2026. Title: RODENTICIDE. Applicant: PelGen Limited. The sequence listing filed with the application follows.

SEQUENCE LISTING (10 sequences)

SEQ ID NO: 1 - protein, 17 aa, Synthetic construct
LKCHNKLVIPXVAWYKT

SEQ ID NO: 2 - protein, 13 aa, synthetic construct
LKCHKLVPPVWKT

SEQ ID NO: 3 - protein, 13 aa, synthetic construct
LKCNKLIPLAYKT

SEQ ID NO: 4 - protein, 14 aa, synthetic construct
LKCHKLIPIAWKTK

SEQ ID NO: 5 - protein, 60 aa, synthetic construct
LKCHKLVPPVWKTCPEGKNLCYKMFMVSTSTVPVKRGCIDVCPKDSALVKYVCCSTDKCN

SEQ ID NO: 6 - protein, 60 aa, synthetic construct
LKCNKLIPLAYKTCPAGKDLCYKMYMVSDKTVPVKRGCIDVCPKNSLLVKYECCNTDRCN

SEQ ID NO: 7 - protein, 60 aa, synthetic construct
LKCNKLVPLFYKTCPAGKDLCYKMYMVATPKVPVKRGCIDVCPKSSLLVKYVCCNTDRCN

SEQ ID NO: 8 - protein, 60 aa, synthetic construct
LKCNQLIPPFWKTCPKGKNLCYKMTMRAAPMVPVKRGCIDVCPKSSLLIKYMCCNTDKCN

SEQ ID NO: 9 - protein, 60 aa, synthetic construct
LKCNKLIPIAYKTCPEGKNLCYKMMLASKKMVPVKRGCIDVCPKDSALVKYVCCSTDRCN

SEQ ID NO: 10 - protein, 60 aa, synthetic construct
LKCNKLVPLFYKTCPAGKNLCYKMFMVSNLTVPVKRGCIDVCPKSSLLVKYVCCNTDRCN